European Patent Application EP 4 772 198 A2, published July 8, 2026. Title: BINDING MOLECULES TO TUMOR ASSOCIATED MACROPHAGES AND METHODS OF USE. Applicant: Sanford Burnham Prebys Medical Discovery Institute. The sequence listing filed with the application follows.

SEQUENCE LISTING (2 sequences)

SEQ ID NO: 1 - protein, 9 aa, synthetic construct
  REGION 1..9: note = Description of Artificial Sequence: Synthetic peptide
CRVLRSGSC

SEQ ID NO: 2 - protein, 8 aa, synthetic construct
  REGION 1..8: note = Description of Artificial Sequence: Synthetic peptide
GGSGGSKG